European Patent Application EP 4 253 570 A2, published October 4, 2023. Title: Escherichia Coli-Based Recombinant Strain, Construction Method and Use Thereof. Applicant: Inner Mongolia Eppen Biotech Co Ltd. The sequence listing filed with the application follows.

SEQUENCE LISTING (22 sequences)

SEQ ID NO: 1 - DNA, 1224 bp, Escherichia coli
  source 1..1224: mol_type = genomic DNA
atgaaacgtgcatttattatggtgctggactcattcggcatcggcgctacagaagatgcagaacgctttggtgacgtcggggctgacaccctgggtcatatcgcagaagcttgtgccaaaggcgaagctgataacggtcgtaaaggcccgctcaatctgccaaatctgacccgtctggggctggcgaaagcacacgaaggttctaccggtttcattccggcgggaatggacggcaacgctgaagttatcggcgcgtacgcatgggcgcacgaaatgtcatccggtaaagataccccgtctggtcactgggaaattgccggtgtcccggttctgtttgagtggggatatttctccgatcacgaaaacagcttcccgcaagagctgctggataaactggtcgaacgcgctaatctgccgggttacctcggtaactgccactcttccggtacggtcattctggatcaactgggcgaagagcacatgaaaaccggcaagccgattttctatacctccgctgactccgtgttccagattgcctgccatgaagaaactttcggtctggataaactctacgaactgtgcgaaatcgcccgtgaagagctgaccaacggcggctacaatatcggtcgtgttatcgctcgtccgtttatcggcgacaaagccggtaacttccagcgtaccggtaaccgtcacgacctggctgttgagccgccagcaccgaccgtgctgcagaaactggttgatgaaaaacacggccaggtggtttctgtcggtaaaattgcggacatctacgccaactgcggtatcaccaaaaaagtgaaagcgactggcctggacgcgctgtttgacgccaccatcaaagagatgaaagaagcgggtgataacaccatcgtcttcaccaacttcgttgacttcgactcttcctggggccaccgtcgcgacgtcgccggttatgccgcgggtctggaactgttcgaccgccgtctgccggagctgatgtctctgctgcgcgatgacgacatcctgatcctcaccgctgaccacggttgcgatccgacctggaccggtactgaccacacgcgtgaacacattccggtactggtatatggcccgaaagtaaaaccgggctcactgggtcatcgtgaaaccttcgcggatatcggccagactctggcaaaatattttggtacttctgatatggaatatggcaaagccatgttctga

SEQ ID NO: 2 - DNA, 1224 bp, synthetic construct
  source 1..1224: mol_type = other DNA
atgaaacgtgcatttattatggtgctggactcattcggcatcggcgctacagaagatgcagaacgctttggtgacgtcggggctgacaccctgggtcatatcgcagaagcttgtgccaaaggcgaagctgataacggtcgtaaaggcccgctcaatctgccaaatctgacccgtctggggctggcgaaagcacacgaaggttctaccggtttcattccggcgggaatggacggcaacgctgaagttatcggcgcgtacgcatgggcgcacgaaatgtcatccggtaaagataccccgtctggtcactgggaaattgccggtgtcccggttctgtttgagtggggatatttctccgatcacgaaaacagcttcccgcaagagctgctggataaactggtcgaacgcgctaatctgccgggttacctcggtaactgccactcttccggtacggtcattctggatcaactgggcgaagagcacatgaaaaccggcaagccgattttctatacctccgctgactccgtgttccagattgcctgccatgaagaaactttcggtctggataaactctacgaactgtgcgaaatcgcccgtgaagagctgaccaacggcggctacaatatcggtcgtgttatcgctcgtccgtttatcggcgacaaagccggtaacttccagcgtaccggtaaccgtcacgacctggctgttgagccgccagcaccgaccgtgctgcagaaactggttgatgaaaaacacggccaggtggtttctgtcggtaaaattgcggacatctacgccaactgcggtatcaccaaaaaagtgaaagcgactggcctggacgcgctgtttgacgccaccatcaaagagatgaaagaagcgggtgataacaccatcgtcttcaccaacttcgttgacttcgactcttcctggggccaccgtcgcgacgtcgccggttatgccgcgggtctggaactgttcgaccgccgtctgccggagctgatgtctctgctgcgcgatgacgacatcctgatcctcaccgctgaccacggttacgatccgacctggaccggtactgaccacacgcgtgaacacattccggtactggtatatggcccgaaagtaaaaccgggctcactgggtcatcgtgaaaccttcgcggatatcggccagactctggcaaaatattttggtacttctgatatggaatatggcaaagccatgttctga

SEQ ID NO: 3 - protein, 407 aa, Escherichia coli
MKRAFIMVLDSFGIGATEDAERFGDVGADTLGHIAEACAKGEADNGRKGPLNLPNLTRLGLAKAHEGSTGFIPAGMDGNAEVIGAYAWAHEMSSGKDTPSGHWEIAGVPVLFEWGYFSDHENSFPQELLDKLVERANLPGYLGNCHSSGTVILDQLGEEHMKTGKPIFYTSADSVFQIACHEETFGLDKLYELCEIAREELTNGGYNIGRVIARPFIGDKAGNFQRTGNRHDLAVEPPAPTVLQKLVDEKHGQVVSVGKIADIYANCGITKKVKATGLDALFDATIKEMKEAGDNTIVFTNFVDFDSSWGHRRDVAGYAAGLELFDRRLPELMSLLRDDDILILTADHGCDPTWTGTDHTREHIPVLVYGPKVKPGSLGHRETFADIGQTLAKYFGTSDMEYGKAMF

SEQ ID NO: 4 - protein, 407 aa, synthetic construct
MKRAFIMVLDSFGIGATEDAERFGDVGADTLGHIAEACAKGEADNGRKGPLNLPNLTRLGLAKAHEGSTGFIPAGMDGNAEVIGAYAWAHEMSSGKDTPSGHWEIAGVPVLFEWGYFSDHENSFPQELLDKLVERANLPGYLGNCHSSGTVILDQLGEEHMKTGKPIFYTSADSVFQIACHEETFGLDKLYELCEIAREELTNGGYNIGRVIARPFIGDKAGNFQRTGNRHDLAVEPPAPTVLQKLVDEKHGQVVSVGKIADIYANCGITKKVKATGLDALFDATIKEMKEAGDNTIVFTNFVDFDSSWGHRRDVAGYAAGLELFDRRLPELMSLLRDDDILILTADHGYDPTWTGTDHTREHIPVLVYGPKVKPGSLGHRETFADIGQTLAKYFGTSDMEYGKAMF

SEQ ID NO: 5 - DNA, 27 bp, synthetic construct
  source 1..27: mol_type = other DNA
cgggatccatggacggcaacgctgaag

SEQ ID NO: 6 - DNA, 18 bp, synthetic construct
  source 1..18: mol_type = other DNA
gatcgtaaccgtggtcag

SEQ ID NO: 7 - DNA, 18 bp, synthetic construct
  source 1..18: mol_type = other DNA
ctgaccacggttacgatc

SEQ ID NO: 8 - DNA, 36 bp, synthetic construct
  source 1..36: mol_type = other DNA
aaggaaaaaagcggccgcgctcgtgagtgcggatgt

SEQ ID NO: 9 - DNA, 20 bp, synthetic construct
  source 1..20: mol_type = other DNA
tgacgccaccatcaaagaga

SEQ ID NO: 10 - DNA, 19 bp, synthetic construct
  source 1..19: mol_type = other DNA
gtcaacgctccgcccaaat

SEQ ID NO: 11 - DNA, 1684 bp, synthetic construct
  source 1..1684: mol_type = other DNA
gacggcaacgctgaagttatcggcgcgtacgcatgggcgcacgaaatgtcatccggtaaagataccccgtctggtcactgggaaattgccggtgtcccggttctgtttgagtggggatatttctccgatcacgaaaacagcttcccgcaagagctgctggataaactggtcgaacgcgctaatctgccgggttacctcggtaactgccactcttccggtacggtcattctggatcaactgggcgaagagcacatgaaaaccggcaagccgattttctatacctccgctgactccgtgttccagattgcctgccatgaagaaactttcggtctggataaactctacgaactgtgcgaaatcgcccgtgaagagctgaccaacggcggctacaatatcggtcgtgttatcgctcgtccgtttatcggcgacaaagccggtaacttccagcgtaccggtaaccgtcacgacctggctgttgagccgccagcaccgaccgtgctgcagaaactggttgatgaaaaacacggccaggtggtttctgtcggtaaaattgcggacatctacgccaactgcggtatcaccaaaaaagtgaaagcgactggcctggacgcgctgtttgacgccaccatcaaagagatgaaagaagcgggtgataacaccatcgtcttcaccaacttcgttgacttcgactcttcctggggccaccgtcgcgacgtcgccggttatgccgcgggtctggaactgttcgaccgccgtctgccggagctgatgtctctgctgcgcgatgacgacatcctgatcctcaccgctgaccacggttacgatccgacctggaccggtactgaccacacgcgtgaacacattccggtactggtatatggcccgaaagtaaaaccgggctcactgggtcatcgtgaaaccttcgcggatatcggccagactctggcaaaatattttggtacttctgatatggaatatggcaaagccatgttctgatggatttgggcggagcgttgactccgcctttgttatgtcacaaaaaggataaaacaatggctaccccacacattaatgcagaaatgggcgatttcgctgacgtagttttgatgccaggcgacccgctgcgtgcgaagtatattgctgaaactttccttgaagatgcccgtgaagtgaacaacgttcgcggtatgctgggcttcaccggtacttacaaaggccgcaaaatttccgtaatgggtcacggtatgggtatcccgtcctgctccatctacaccaaagaactgatcaccgatttcggcgtgaagaaaattatccgcgtgggttcctgtggcgcagttctgccgcacgtaaaactgcgcgacgtcgttatcggtatgggtgcctgcaccgattccaaagttaaccgcatccgttttaaagaccatgactttgccgctatcgctgacttcgacatggtgcgtaacgcagtagatgcagctaaagcactgggtattgatgctcgcgtgggtaacctgttctccgctgacctgttctactctccggacggcgaaatgttcgacgtgatggaaaaatacggcattctcggcgtggaaatggaagcggctggtatctacggcgtcgctgcagaatttggcgcgaaagccctgaccatctgcaccgtatctgaccacatccgcactcacga

SEQ ID NO: 12 - DNA, 401 bp, synthetic construct
  source 1..401: mol_type = other DNA
tgacgccaccatcaaagagatgaaagaagcgggtgataacaccatcgtcttcaccaacttcgttgacttcgactcttcctggggccaccgtcgcgacgtcgccggttatgccgcgggtctggaactgttcgaccgccgtctgccggagctgatgtctctgctgcgcgatgacgacatcctgatcctcaccgctgaccacggttacgatccgacctggaccggtactgaccacacgcgtgaacacattccggtactggtatatggcccgaaagtaaaaccgggctcactgggtcatcgtgaaaccttcgcggatatcggccagactctggcaaaatattttggtacttctgatatggaatatggcaaagccatgttctgatggatttgggcggagcgttgac

SEQ ID NO: 13 - DNA, 355 bp, Escherichia coli
  source 1..355: mol_type = genomic DNA
cataaccacctcaaatgtgattcaaataagtcctaagttttaaatatatcaaaaattaatgggaaactcttcgcgatttgtgatgtctaacgggccatttcatgtaacagaacgtttccatacaccgctatccatctaaatttaaatcactttttcagagaactgcgtaagtattacgcatgttttccctgtcattcatccagattattcctaatcaccagactaatgattccatcaatcctggcgcattttagtcaaaacgggggaaaattttttcaacaaatgctcaaccagcattgggtatatccagtacactccacgctttacttaagtctagatatttgtgggagaaagg

SEQ ID NO: 14 - DNA, 355 bp, synthetic construct
  source 1..355: mol_type = other DNA
cataaccacctcaaatgtgattcaaataagtcctaagttttaaatatatcaaaaattaatgggaaactcttcgcgatttgtgatgtctaacgggccatttcatgtaacagaacgtttccatacaccgctatccatctaaatttaaatcactttttcagagaactgcgtaagtattacgcatgttttccctgtcattcatccagattattcctaatcaccagactaatgattccatcaatcctggcgcattttagtcaaaacgggggaaaattttttcaacaaatgctcgaccagcattgggtatatccagtacactccacgctttacttaagtctagatatttgtgggagaaagg

SEQ ID NO: 15 - DNA, 888 bp, Escherichia coli
  source 1..888: mol_type = genomic DNA
atgcctggttcattacgtaaaatgccggtctggttaccaatagtcatattgctcgttgccatggcgtctattcagggtggagcctcgttagctaagtcactttttcctctggtgggcgcaccgggtgtcactgcgctgcgtctggcattaggaacgctgatcctcatcgcgttctttaagccatggcgactgcgctttgccaaagagcaacggttaccgctgttgttttacggcgtttcgctgggtgggatgaattatcttttttatctttctattcagacagtaccgctgggtattgcggtggcgctggagttcaccggaccactggcggtggcgctgttctcttctcgtcgcccggtagatttcgtctgggttgtgctggcggttcttggtctgtggttcctgctaccgctggggcaagacgtttcccatgtcgatttaaccggctgtgcgctggcactgggggccggggcttgttgggctatttacattttaagtgggcaacgcgcaggagcggaacatggccctgcgacggtggcaattggttcgttgattgcagcgttaattttcgtgccaattggagcgcttcaggctggtgaagcactctggcactggtcggttattccattgggtctggctgtcgctattctctcgaccgctctgccttattcgctggaaatgattgccctcacccgtttgccaacacggacatttggtacgctgatgagcatggaaccggcgctggctgccgtttccgggatgattttcctcggagaaacactgacacccatacagctactggcgctcggcgctatcatcgccgcttcaatggggtctacgctgacagtacgcaaagagagcaaaataaaagaattagacattaattaa

SEQ ID NO: 16 - protein, 295 aa, Escherichia coli
MPGSLRKMPVWLPIVILLVAMASIQGGASLAKSLFPLVGAPGVTALRLALGTLILIAFFKPWRLRFAKEQRLPLLFYGVSLGGMNYLFYLSIQTVPLGIAVALEFTGPLAVALFSSRRPVDFVWVVLAVLGLWFLLPLGQDVSHVDLTGCALALGAGACWAIYILSGQRAGAEHGPATVAIGSLIAALIFVPIGALQAGEALWHWSVIPLGLAVAILSTALPYSLEMIALTRLPTRTFGTLMSMEPALAAVSGMIFLGETLTPIQLLALGAIIAASMGSTLTVRKESKIKELDIN

SEQ ID NO: 17 - DNA, 30 bp, synthetic construct
  source 1..30: mol_type = other DNA
cgggatcctcgctggtgtcgtgtttgtagg

SEQ ID NO: 18 - DNA, 20 bp, synthetic construct
  source 1..20: mol_type = other DNA
tatacccaatgctggtcgag

SEQ ID NO: 19 - DNA, 20 bp, synthetic construct
  source 1..20: mol_type = other DNA
cgaccagcattgggtatatc

SEQ ID NO: 20 - DNA, 41 bp, synthetic construct
  source 1..41: mol_type = other DNA
aaggaaaaaagcggccgccgaaaattaacgctgcaatcaac

SEQ ID NO: 21 - DNA, 18 bp, synthetic construct
  source 1..18: mol_type = other DNA
atacaccgctatccatct

SEQ ID NO: 22 - DNA, 18 bp, synthetic construct
  source 1..18: mol_type = other DNA
aaccaggcatcctttctc